European Patent Specification EP 3 555 123 B1, published March 27, 2024. Title: COMPOSITION COMPRISING RECOMBINANT GpIba RECEPTOR PROTEIN. Applicant: GRIFOLS DIAGNOSTIC SOLUTIONS INC. The sequence listing filed with the application follows.

SEQUENCE LISTING (46 sequences)

SEQ ID NO: 1 - protein, 290 aa, Synthetic
HPICEVSKVASHLEVNCDKRNLTALPPDLPKDTTILHLSENLLYTFSLATLMPYTRLTQLNLDRSELTKLQVDGTLPVLGTLDLSHNQLQSLPLLGQTLPALTVLDVSFNRLTSLPLGALRGLGELQELYLKGNELKTLPPGLLTPTPKLEKLSLANNNLTELPAGLLNGLENLDTLLLQENSLYTIPKGFFGSHLLPFAFLHGNPWLCNCEILYFRRWLQDNAENVYVWKQGVDVKAMTSNVASVQCDNSDKFPVYKYPGKGCPTLGDEGDTDLYDYYPEEDTEGDKVR

SEQ ID NO: 2 - protein, 290 aa, Synthetic
HPICEVSKVASHLEVNCDKRNLTALPPDLPKDTTILHLSENLLYTFSLATLMPYTRLTQLNLDRSELTKLQVDGTLPVLGTLDLSHNQLQSLPLLGQTLPALTVLDVSFNRLTSLPLGALRGLGELQELYLKGNELKTLPPGLLTPTPKLEKLSLANNNLTELPAGLLNGLENLDTLLLQENSLYTIPKGFFGSHLLPFAFLHGNPWLCNCEILYFRRWLQDNAENVYVWKQGVVVKAMTSNVASVQCDNSDKFPVYKYPGKGCPTLGDEGDTDLYDYYPEEDTEGDKVR

SEQ ID NO: 3 - protein, 290 aa, Synthetic
HPICEVSKVASHLEVNCDKRNLTALPPDLPKDTTILHLSENLLYTFSLATLMPYTRLTQLNLDRSELTKLQVDGTLPVLGTLDLSHNQLQSLPLLGQTLPALTVLDVSFNRLTSLPLGALRGLGELQELYLKGNELKTLPPGLLTPTPKLEKLSLANNNLTELPAGLLNGLENLDTLLLQENSLYTIPKGFFGSHLLPFAFLHGNPWLCNCEILYFRRWLQDNAENVYVWKQGVDVVAMTSNVASVQCDNSDKFPVYKYPGKGCPTLGDEGDTDLYDYYPEEDTEGDKVR

SEQ ID NO: 4 - protein, 290 aa, Synthetic
HPICEVSKVASHLEVNCDKRNLTALPPDLPKDTTILHLSENLLYTFSLATLMPYTRLTQLNLDRSELTKLQVDGTLPVLGTLDLSHNQLQSLPLLGQTLPALTVLDVSFNRLTSLPLGALRGLGELQELYLKGNELKTLPPGLLTPTPKLEKLSLANNNLTELPAGLLNGLENLDTLLLQENSLYTIPKGFFGSHLLPFAFLHGNPWLCNCEILYFRRWLQDNAENVYVWKQTVDVKAMTSNVASVQCDNSDKFPVYKYPGKGCPTLGDEGDTDLYDYYPEEDTEGDKVR

SEQ ID NO: 5 - protein, 290 aa, Synthetic
HPICEVSKVASHLEVNCDKRNLTALPPDLPKDTTILHLSENLLYTFSLATLMPYTRLTQLNLDRSELTKLQVDGTLPVLGTLDLSHNQLQSLPLLGQTLPALTVLDVSFNRLTSLPLGALRGLGELQELYLKGNELKTLPPGLLTPTPKLEKLSLANNNLTELPAGLLNGLENLDTLLLQENSLYTIPKGFFGSHLLPFAFLHGNPWLCNCEILYFRRWLQDNAENVYVWKQTVDVKATTSNVASVQCDNSDKFPVYKYPGKGCPTLGDEGDTDLYDYYPEEDTEGDKVR

SEQ ID NO: 6 - protein, 290 aa, Synthetic
HPICEVSKVASHLEVNCDKRNLTALPPDLPKDTTILHLSENLLYTFSLATLMPYTRLTQLNLDRSELTKLQVDGTLPVLGTLDLSHNQLQSLPLLGQTLPALTVLDVSFNRLTSLPLGALRGLGELQELYLKGNELKTLPPGLLTPTPKLEKLSLANNNLTELPAGLLNGLENLDTLLLQENSLYTIPKGFFGSHLLPFAFLHGNPWLCNCEILYFRRWLQDNAENVYVWKQGVDVKVMTSNVASVQCDNSDKFPVYKYPGKGCPTLGDEGDTDLYDYYPEEDTEGDKVR

SEQ ID NO: 7 - protein, 290 aa, Synthetic
HPICEVSKVASHLEVNCDKRNLTALPPDLPKDTTILHLSENLLYTFSLATLMPYTRLTQLNLDRSELTKLQVDGTLPVLGTLDLSHNQLQSLPLLGQTLPALTVLDVSFNRLTSLPLGALRGLGELQELYLKGNELKTLPPGLLTPTPKLEKLSLANNNLTELPAGLLNGLENLDTLLLQENSLYTIPKGFFGSHLLPFAFLHGNPWLCNCEILYFRRWLQDNAENVYVWKQVVDVKAMTSNVASVQCDNSDKFPVYKYPGKGCPTLGDEGDTDLYDYYPEEDTEGDKVR

SEQ ID NO: 8 - protein, 290 aa, Synthetic
HPICEVSKVASHLEVNCDKRNLTALPPDLPKDTTILHLSENLLYTFSLATLMPYTRLTQLNLDRSELTKLQVDGTLPVLGTLDLSHNQLQSLPLLGQTLPALTVLDVSFNRLTSLPLGALRGLGELQELYLKGNELKTLPPGLLTPTPKLEKLSLANNNLTELPAGLLNGLENLDTLLLQENSLYTIPKGFFGSHLLPFAFLHGNPWLCNCEILYFRRWLQDNAENVYVWKQVVDVKAVTSNVASVQCDNSDKFPVYKYPGKGCPTLGDEGDTDLYDYYPEEDTEGDKVR

SEQ ID NO: 9 - protein, 278 aa, Synthetic
HPICEVSKVASHLEVNCDKRNLTALPPDLPKDTTILHLSENLLYTFSLATLMPYTRLTQLNLDRSELTKLQVDGTLPVLGTLDLSHNQLQSLPLLGQTLPALTVLDVSFNRLTSLPLGALRGLGELQELYLKGNELKTLPPGLLTPTPKLEKLSLANNNLTELPAGLLNGLENLDTLLLQENSLYTIPKGFFGSHLLPFAFLHGNPWLCNCEILYFRRWLQDNAENVYSNVASVQCDNSDKFPVYKYPGKGCPTLGDEGDTDLYDYYPEEDTEGDKVR

SEQ ID NO: 10 - protein, 40 aa, Synthetic
KPLDGEYFTLQIRGRERFEMFRELNEALELKDAQAGKEPG

SEQ ID NO: 11 - protein, 227 aa, Synthetic
VPRDCGCKPCICTVPEVSSVFIFPPKPKDVLTITLTPKVTCVVVDISKDDPEVQFSWFVDDVEVHTAQTQPREEQFNSTFRSVSELPIMHQDWLNGKEFKCRVNSAAFPAPIEKTISKTKGRPKAPQVYTIPPPKEQMAKDKVSLTCMITDFFPEDITVEWQWNGQPAENYKNTQPIMDTDGSYFVYSKLNVQKSNWEAGNTFTCSVLHEGLHNHHTEKSLSHSPGI

SEQ ID NO: 12 - protein, 231 aa, Synthetic
PRGPTIKPCPPCKCPAPNLLGGPSVFIFPPKIKDVLMISLSPIVTCVVVDVSEDDPDVQISWFVNNVEVHTAQTQTHREDYNSTLRVVSALPIQHQDWMSGKEFKCKVNNKDLPAPIERTISKPKGSVRAPQVYVLPPPEEEMTKKQVTLTCMVTDFMPEDIYVEWTNNGKTELNYKNTEPVLDSDGSYFMYSKLRVEKKNWVERNSYSCSVVHEGLHNHHTTKSFSRTPG

SEQ ID NO: 13 - protein, 27 aa, Synthetic
GYIPEAPRDGQAYVRKDGEWVLLSTFL

SEQ ID NO: 14 - protein, 94 aa, Synthetic
GSHMWKQSVELAKKDSLYKDAMQYASESKDTELAEELLQWFLQEEKRECFGACLFTCYDLLRPDVVLELAWRHNIMDFAMPYFIQVMKEYLTKV

SEQ ID NO: 15 - protein, 6 aa, Synthetic
HHHHHH

SEQ ID NO: 16 - protein, 7 aa, Synthetic
HHHHHHC

SEQ ID NO: 17 - protein, 21 aa, Synthetic
EEAAEEEAAEESDDDHHHHHH

SEQ ID NO: 18 - protein, 44 aa, Synthetic
MDEKTTGWRGGHVVEGLAGELEQLRARLEHHPQGQREPHHHHHH

SEQ ID NO: 19 - protein, 290 aa, Homo sapiens
HPICEVSKVASHLEVNCDKRNLTALPPDLPKDTTILHLSENLLYTFSLATLMPYTRLTQLNLDRCELTKLQVDGTLPVLGTLDLSHNQLQSLPLLGQTLPALTVLDVSFNRLTSLPLGALRGLGELQELYLKGNELKTLPPGLLTPTPKLEKLSLANNNLTELPAGLLNGLENLDTLLLQENSLYTIPKGFFGSHLLPFAFLHGNPWLCNCEILYFRRWLQDNAENVYVWKQGVDVKAMTSNVASVQCDNSDKFPVYKYPGKGCPTLGDEGDTDLYDYYPEEDTEGDKVR

SEQ ID NO: 20 - protein, 25 aa, Homo sapiens
MDAMKRGLCCVLLLCGAVFVSPSAS

SEQ ID NO: 21 - protein, 526 aa, Synthetic
HPICEVSKVASHLEVNCDKRNLTALPPDLPKDTTILHLSENLLYTFSLATLMPYTRLTQLNLDRSELTKLQVDGTLPVLGTLDLSHNQLQSLPLLGQTLPALTVLDVSFNRLTSLPLGALRGLGELQELYLKGNELKTLPPGLLTPTPKLEKLSLANNNLTELPAGLLNGLENLDTLLLQENSLYTIPKGFFGSHLLPFAFLHGNPWLCNCEILYFRRWLQDNAENVYVWKQTVDVKAMTSNVASVQCDNSDKFPVYKYPGKGCPTLGDEGDTDLYDYYPEEDTEGDKVRVPRDCGCKPCICTVPEVSSVFIFPPKPKDVLTITLTPKVTCVVVDISKDDPEVQFSWFVDDVEVHTAQTQPREEQFNSTFRSVSELPIMHQDWLNGKEFKCRVNSAAFPAPIEKTISKTKGRPKAPQVYTIPPPKEQMAKDKVSLTCMITDFFPEDITVEWQWNGQPAENYKNTQPIMDTDGSYFVYSKLNVQKSNWEAGNTFTCSVLHEGLHNHHTEKSLSHSPGIGHHHHHHHH

SEQ ID NO: 22 - protein, 336 aa, Synthetic
HPICEVSKVASHLEVNCDKRNLTALPPDLPKDTTILHLSENLLYTFSLATLMPYTRLTQLNLDRSELTKLQVDGTLPVLGTLDLSHNQLQSLPLLGQTLPALTVLDVSFNRLTSLPLGALRGLGELQELYLKGNELKTLPPGLLTPTPKLEKLSLANNNLTELPAGLLNGLENLDTLLLQENSLYTIPKGFFGSHLLPFAFLHGNPWLCNCEILYFRRWLQDNAENVYVWKQTVDVKAMTSNVASVQCDNSDKFPVYKYPGKGCPTLGDEGDTDLYDYYPEEDTEGDKVRKPLDGEYFTLQIRGRERFEMFRELNEALELKDAQAGKEPGHHHHHH

SEQ ID NO: 23 - protein, 336 aa, Synthetic
HPICEVSKVASHLEVNCDKRNLTALPPDLPKDTTILHLSENLLYTFSLATLMPYTRLTQLNLDRSELTKLQVDGTLPVLGTLDLSHNQLQSLPLLGQTLPALTVLDVSFNRLTSLPLGALRGLGELQELYLKGNELKTLPPGLLTPTPKLEKLSLANNNLTELPAGLLNGLENLDTLLLQENSLYTIPKGFFGSHLLPFAFLHGNPWLCNCEILYFRRWLQDNAENVYVWKQVVDVKAVTSNVASVQCDNSDKFPVYKYPGKGCPTLGDEGDTDLYDYYPEEDTEGDKVRKPLDGEYFTLQIRGRERFEMFRELNEALELKDAQAGKEPGHHHHHH

SEQ ID NO: 24 - protein, 297 aa, Synthetic
HPICEVSKVASHLEVNCDKRNLTALPPDLPKDTTILHLSENLLYTFSLATLMPYTRLTQLNLDRSELTKLQVDGTLPVLGTLDLSHNQLQSLPLLGQTLPALTVLDVSFNRLTSLPLGALRGLGELQELYLKGNELKTLPPGLLTPTPKLEKLSLANNNLTELPAGLLNGLENLDTLLLQENSLYTIPKGFFGSHLLPFAFLHGNPWLCNCEILYFRRWLQDNAENVYVWKQTVDVKAMTSNVASVQCDNSDKFPVYKYPGKGCPTLGDEGDTDLYDYYPEEDTEGDKVRHHHHHHC

SEQ ID NO: 25 - protein, 334 aa, Synthetic
HPICEVSKVASHLEVNCDKRNLTALPPDLPKDTTILHLSENLLYTFSLATLMPYTRLTQLNLDRSELTKLQVDGTLPVLGTLDLSHNQLQSLPLLGQTLPALTVLDVSFNRLTSLPLGALRGLGELQELYLKGNELKTLPPGLLTPTPKLEKLSLANNNLTELPAGLLNGLENLDTLLLQENSLYTIPKGFFGSHLLPFAFLHGNPWLCNCEILYFRRWLQDNAENVYVWKQTVDVKAMTSNVASVQCDNSDKFPVYKYPGKGCPTLGDEGDTDLYDYYPEEDTEGDKVRMDEKTTGWRGGHVVEGLAGELEQLRARLEHHPQGQREPHHHHHH

SEQ ID NO: 26 - protein, 336 aa, Synthetic
HPICEVSKVASHLEVNCDKRNLTALPPDLPKDTTILHLSENLLYTFSLATLMPYTRLTQLNLDRAELTKLQVDGTLPVLGTLDLSHNQLQSLPLLGQTLPALTVLDVSFNRLTSLPLGALRGLGELQELYLKGNELKTLPPGLLTPTPKLEKLSLANNNLTELPAGLLNGLENLDTLLLQENSLYTIPKGFFGSHLLPFAFLHGNPWLCNCEILYFRRWLQDNAENVYVWKQVVDVKAVTSNVASVQCDNSDKFPVYKYPGKGCPTLGDEGDTDLYDYYPEEDTEGDKVRKPLDGEYFTLQIRGRERFEMFRELNEALELKDAQAGKEPGHHHHHH

SEQ ID NO: 27 - protein, 296 aa, Synthetic
HPICEVSKVASHLEVNCDKRNLTALPPDLPKDTTILHLSENLLYTFSLATLMPYTRLTQLNLDRAELTKLQVDGTLPVLGTLDLSHNQLQSLPLLGQTLPALTVLDVSFNRLTSLPLGALRGLGELQELYLKGNELKTLPPGLLTPTPKLEKLSLANNNLTELPAGLLNGLENLDTLLLQENSLYTIPKGFFGSHLLPFAFLHGNPWLCNCEILYFRRWLQDNAENVYVWKQVVDVKAVTSNVASVQCDNSDKFPVYKYPGKGCPTLGDEGDTDLYDYYPEEDTEGDKVRHHHHHH

SEQ ID NO: 28 - protein, 308 aa, Synthetic
HPICEVSKVASHLEVNCDKRNLTALPPDLPKDTTILHLSENLLYTFSLATLMPYTRLTQLNLDRAELTKLQVDGTLPVLGTLDLSHNQLQSLPLLGQTLPALTVLDVSFNRLTSLPLGALRGLGELQELYLKGNELKTLPPGLLTPTPKLEKLSLANNNLTELPAGLLNGLENLDTLLLQENSLYTIPKGFFGSHLLPFAFLHGNPWLCNCEILYFRRWLQDNAENVYVWKQVVDVKAVTSNVASVQCDNSDKFPVYKYPGKGCPTLGDEGDTDLYDYYPEEDTEGDEEAAEEEAAEESDDDHHHHHH

SEQ ID NO: 29 - protein, 313 aa, Synthetic
HPICEVSKVASHLEVNCDKRNLTALPPDLPKDTTILHLSENLLYTFSLATLMPYTRLTQLNLDRCELTKLQVDGTLPVLGTLDLSHNQLQSLPLLGQTLPALTVLDVSFNRLTSLPLGALRGLGELQELYLKGNELKTLPPGLLTPTPKLEKLSLANNNLTELPAGLLNGLENLDTLLLQENSLYTIPKGFFGSHLLPFAFLHGNPWLCNCEILYFRRWLQDNAENVYVWKQVVDVKAVTSNVASVQCDNSDKFPVYKYPGKGCPTLGDEGDTDLYDYYPEEDTEDYKDHDGDYKDHDIDYKDDDDKHHHHHH

SEQ ID NO: 30 - protein, 526 aa, Synthetic
HPICEVSKVASHLEVNCDKRNLTALPPDLPKDTTILHLSENLLYTFSLATLMPYTRLTQLNLDRSELTKLQVDGTLPVLGTLDLSHNQLQSLPLLGQTLPALTVLDVSFNRLTSLPLGALRGLGELQELYLKGNELKTLPPGLLTPTPKLEKLSLANNNLTELPAGLLNGLENLDTLLLQENSLYTIPKGFFGSHLLPFAFLHGNPWLCNCEILYFRRWLQDNAENVYVWKQGVVVKAMTSNVASVQCDNSDKFPVYKYPGKGCPTLGDEGDTDLYDYYPEEDTEGDKVRVPRDCGCKPCICTVPEVSSVFIFPPKPKDVLTITLTPKVTCVVVDISKDDPEVQFSWFVDDVEVHTAQTQPREEQFNSTFRSVSELPIMHQDWLNGKEFKCRVNSAAFPAPIEKTISKTKGRPKAPQVYTIPPPKEQMAKDKVSLTCMITDFFPEDITVEWQWNGQPAENYKNTQPIMDTDGSYFVYSKLNVQKSNWEAGNTFTCSVLHEGLHNHHTEKSLSHSPGIGHHHHHHHH

SEQ ID NO: 31 - protein, 526 aa, Synthetic
HPICEVSKVASHLEVNCDKRNLTALPPDLPKDTTILHLSENLLYTFSLATLMPYTRLTQLNLDRSELTKLQVDGTLPVLGTLDLSHNQLQSLPLLGQTLPALTVLDVSFNRLTSLPLGALRGLGELQELYLKGNELKTLPPGLLTPTPKLEKLSLANNNLTELPAGLLNGLENLDTLLLQENSLYTIPKGFFGSHLLPFAFLHGNPWLCNCEILYFRRWLQDNAENVYVWKQGVDVVAMTSNVASVQCDNSDKFPVYKYPGKGCPTLGDEGDTDLYDYYPEEDTEGDKVRVPRDCGCKPCICTVPEVSSVFIFPPKPKDVLTITLTPKVTCVVVDISKDDPEVQFSWFVDDVEVHTAQTQPREEQFNSTFRSVSELPIMHQDWLNGKEFKCRVNSAAFPAPIEKTISKTKGRPKAPQVYTIPPPKEQMAKDKVSLTCMITDFFPEDITVEWQWNGQPAENYKNTQPIMDTDGSYFVYSKLNVQKSNWEAGNTFTCSVLHEGLHNHHTEKSLSHSPGIGHHHHHHHH

SEQ ID NO: 32 - protein, 526 aa, Synthetic
HPICEVSKVASHLEVNCDKRNLTALPPDLPKDTTILHLSENLLYTFSLATLMPYTRLTQLNLDRSELTKLQVDGTLPVLGTLDLSHNQLQSLPLLGQTLPALTVLDVSFNRLTSLPLGALRGLGELQELYLKGNELKTLPPGLLTPTPKLEKLSLANNNLTELPAGLLNGLENLDTLLLQENSLYTIPKGFFGSHLLPFAFLHGNPWLCNCEILYFRRWLQDNAENVYVWKQVVDVKAMTSNVASVQCDNSDKFPVYKYPGKGCPTLGDEGDTDLYDYYPEEDTEGDKVRVPRDCGCKPCICTVPEVSSVFIFPPKPKDVLTITLTPKVTCVVVDISKDDPEVQFSWFVDDVEVHTAQTQPREEQFNSTFRSVSELPIMHQDWLNGKEFKCRVNSAAFPAPIEKTISKTKGRPKAPQVYTIPPPKEQMAKDKVSLTCMITDFFPEDITVEWQWNGQPAENYKNTQPIMDTDGSYFVYSKLNVQKSNWEAGNTFTCSVLHEGLHNHHTEKSLSHSPGIGHHHHHHHH

SEQ ID NO: 33 - protein, 526 aa, Synthetic
HPICEVSKVASHLEVNCDKRNLTALPPDLPKDTTILHLSENLLYTFSLATLMPYTRLTQLNLDRSELTKLQVDGTLPVLGTLDLSHNQLQSLPLLGQTLPALTVLDVSFNRLTSLPLGALRGLGELQELYLKGNELKTLPPGLLTPTPKLEKLSLANNNLTELPAGLLNGLENLDTLLLQENSLYTIPKGFFGSHLLPFAFLHGNPWLCNCEILYFRRWLQDNAENVYVWKQTVDVKATTSNVASVQCDNSDKFPVYKYPGKGCPTLGDEGDTDLYDYYPEEDTEGDKVRVPRDCGCKPCICTVPEVSSVFIFPPKPKDVLTITLTPKVTCVVVDISKDDPEVQFSWFVDDVEVHTAQTQPREEQFNSTFRSVSELPIMHQDWLNGKEFKCRVNSAAFPAPIEKTISKTKGRPKAPQVYTIPPPKEQMAKDKVSLTCMITDFFPEDITVEWQWNGQPAENYKNTQPIMDTDGSYFVYSKLNVQKSNWEAGNTFTCSVLHEGLHNHHTEKSLSHSPGIGHHHHHHHH

SEQ ID NO: 34 - protein, 526 aa, Synthetic
HPICEVSKVASHLEVNCDKRNLTALPPDLPKDTTILHLSENLLYTFSLATLMPYTRLTQLNLDRSELTKLQVDGTLPVLGTLDLSHNQLQSLPLLGQTLPALTVLDVSFNRLTSLPLGALRGLGELQELYLKGNELKTLPPGLLTPTPKLEKLSLANNNLTELPAGLLNGLENLDTLLLQENSLYTIPKGFFGSHLLPFAFLHGNPWLCNCEILYFRRWLQDNAENVYVWKQVVDVKAVTSNVASVQCDNSDKFPVYKYPGKGCPTLGDEGDTDLYDYYPEEDTEGDKVRVPRDCGCKPCICTVPEVSSVFIFPPKPKDVLTITLTPKVTCVVVDISKDDPEVQFSWFVDDVEVHTAQTQPREEQFNSTFRSVSELPIMHQDWLNGKEFKCRVNSAAFPAPIEKTISKTKGRPKAPQVYTIPPPKEQMAKDKVSLTCMITDFFPEDITVEWQWNGQPAENYKNTQPIMDTDGSYFVYSKLNVQKSNWEAGNTFTCSVLHEGLHNHHTEKSLSHSPGIGHHHHHHHH

SEQ ID NO: 35 - protein, 296 aa, Synthetic
HPICEVSKVASHLEVNCDKRNLTALPPDLPKDTTILHLSENLLYTFSLATLMPYTRLTQLNLDRSELTKLQVDGTLPVLGTLDLSHNQLQSLPLLGQTLPALTVLDVSFNRLTSLPLGALRGLGELQELYLKGNELKTLPPGLLTPTPKLEKLSLANNNLTELPAGLLNGLENLDTLLLQENSLYTIPKGFFGSHLLPFAFLHGNPWLCNCEILYFRRWLQDNAENVYVWKQVVDVKAVTSNVASVQCDNSDKFPVYKYPGKGCPTLGDEGDTDLYDYYPEEDTEGDKVRHHHHHH

SEQ ID NO: 36 - protein, 526 aa, Synthetic
HPICEVSKVASHLEVNCDKRNLTALPPDLPKDTTILHLSENLLYTFSLATLMPYTRLTQLNLDRSELTKLQVDGTLPVLGTLDLSHNQLQSLPLLGQTLPALTVLDVSFNRLTSLPLGALRGLGELQELYLKGNELKTLPPGLLTPTPKLEKLSLANNNLTELPAGLLNGLENLDTLLLQENSLYTIPKGFFGSHLLPFAFLHGNPWLCNCEILYFRRWLQDNAENVYVWKQGVDVKVMTSNVASVQCDNSDKFPVYKYPGKGCPTLGDEGDTDLYDYYPEEDTEGDKVRVPRDCGCKPCICTVPEVSSVFIFPPKPKDVLTITLTPKVTCVVVDISKDDPEVQFSWFVDDVEVHTAQTQPREEQFNSTFRSVSELPIMHQDWLNGKEFKCRVNSAAFPAPIEKTISKTKGRPKAPQVYTIPPPKEQMAKDKVSLTCMITDFFPEDITVEWQWNGQPAENYKNTQPIMDTDGSYFVYSKLNVQKSNWEAGNTFTCSVLHEGLHNHHTEKSLSHSPGIGHHHHHHHH

SEQ ID NO: 37 - protein, 526 aa, Synthetic
HPICEVSKVASHLEVNCDKRNLTALPPDLPKDTTILHLSENLLYTFSLATLMPYTRLTQLNLDRSELTKLQVDGTLPVLGTLDLSHNQLQSLPLLGQTLPALTVLDVSFNRLTSLPLGALRGLGELQELYLKGNELKTLPPGLLTPTPKLEKLSLANNNLTELPAGLLNGLENLDTLLLQENSLYTIPKGFFGSHLLPFAFLHGNPWLCNCEILYFRRWLQDNAENVYVWKQGVDVKAMTSNVASVQCDNSDKFPVYKYPGKGCPTLGDEGDTDLYDYYPEEDTEGDKVRVPRDCGCKPCICTVPEVSSVFIFPPKPKDVLTITLTPKVTCVVVDISKDDPEVQFSWFVDDVEVHTAQTQPREEQFNSTFRSVSELPIMHQDWLNGKEFKCRVNSAAFPAPIEKTISKTKGRPKAPQVYTIPPPKEQMAKDKVSLTCMITDFFPEDITVEWQWNGQPAENYKNTQPIMDTDGSYFVYSKLNVQKSNWEAGNTFTCSVLHEGLHNHHTEKSLSHSPGIGHHHHHHHH

SEQ ID NO: 38 - protein, 514 aa, Synthetic
HPICEVSKVASHLEVNCDKRNLTALPPDLPKDTTILHLSENLLYTFSLATLMPYTRLTQLNLDRSELTKLQVDGTLPVLGTLDLSHNQLQSLPLLGQTLPALTVLDVSFNRLTSLPLGALRGLGELQELYLKGNELKTLPPGLLTPTPKLEKLSLANNNLTELPAGLLNGLENLDTLLLQENSLYTIPKGFFGSHLLPFAFLHGNPWLCNCEILYFRRWLQDNAENVYSNVASVQCDNSDKFPVYKYPGKGCPTLGDEGDTDLYDYYPEEDTEGDKVRVPRDCGCKPCICTVPEVSSVFIFPPKPKDVLTITLTPKVTCVVVDISKDDPEVQFSWFVDDVEVHTAQTQPREEQFNSTFRSVSELPIMHQDWLNGKEFKCRVNSAAFPAPIEKTISKTKGRPKAPQVYTIPPPKEQMAKDKVSLTCMITDFFPEDITVEWQWNGQPAENYKNTQPIMDTDGSYFVYSKLNVQKSNWEAGNTFTCSVLHEGLHNHHTEKSLSHSPGIGHHHHHHHH

SEQ ID NO: 39 - protein, 529 aa, Synthetic
HPICEVSKVASHLEVNCDKRNLTALPPDLPKDTTILHLSENLLYTFSLATLMPYTRLTQLNLDRSELTKLQVDGTLPVLGTLDLSHNQLQSLPLLGQTLPALTVLDVSFNRLTSLPLGALRGLGELQELYLKGNELKTLPPGLLTPTPKLEKLSLANNNLTELPAGLLNGLENLDTLLLQENSLYTIPKGFFGSHLLPFAFLHGNPWLCNCEILYFRRWLQDNAENVYVWKQTVDVKAMTSNVASVQCDNSDKFPVYKYPGKGCPTLGDEGDTDLYDYYPEEDTEGDKVRPRGPTIKPCPPCKCPAPNLLGGPSVFIFPPKIKDVLMISLSPIVTCVVVDVSEDDPDVQISWFVNNVEVHTAQTQTHREDYNSTLRVVSALPIQHQDWMSGKEFKCKVNNKDLPAPIERTISKPKGSVRAPQVYVLPPPEEEMTKKQVTLTCMVTDFMPEDIYVEWTNNGKTELNYKNTEPVLDSDGSYFMYSKLRVEKKNWVERNSYSCSVVHEGLHNHHTTKSFSRTPGHHHHHHHH

SEQ ID NO: 40 - protein, 323 aa, Synthetic
HPICEVSKVASHLEVNCDKRNLTALPPDLPKDTTILHLSENLLYTFSLATLMPYTRLTQLNLDRSELTKLQVDGTLPVLGTLDLSHNQLQSLPLLGQTLPALTVLDVSFNRLTSLPLGALRGLGELQELYLKGNELKTLPPGLLTPTPKLEKLSLANNNLTELPAGLLNGLENLDTLLLQENSLYTIPKGFFGSHLLPFAFLHGNPWLCNCEILYFRRWLQDNAENVYVWKQTVDVKAMTSNVASVQCDNSDKFPVYKYPGKGCPTLGDEGDTDLYDYYPEEDTEGDKVRGYIPEAPRDGQAYVRKDGEWVLLSTFLHHHHHH

SEQ ID NO: 41 - protein, 390 aa, Synthetic
HPICEVSKVASHLEVNCDKRNLTALPPDLPKDTTILHLSENLLYTFSLATLMPYTRLTQLNLDRSELTKLQVDGTLPVLGTLDLSHNQLQSLPLLGQTLPALTVLDVSFNRLTSLPLGALRGLGELQELYLKGNELKTLPPGLLTPTPKLEKLSLANNNLTELPAGLLNGLENLDTLLLQENSLYTIPKGFFGSHLLPFAFLHGNPWLCNCEILYFRRWLQDNAENVYVWKQTVDVKAMTSNVASVQCDNSDKFPVYKYPGKGCPTLGDEGDTDLYDYYPEEDTEGDKVRGSHMWKQSVELAKKDSLYKDAMQYASESKDTELAEELLQWFLQEEKRECFGACLFTCYDLLRPDVVLELAWRHNIMDFAMPYFIQVMKEYLTKVHHHHHH

SEQ ID NO: 42 - protein, 290 aa, Synthetic
HPICEVSKVASHLEVNCDKRNLTALPPDLPKDTTILHLSENLLYTFSLATLMPYTRLTQLNLDRAELTKLQVDGTLPVLGTLDLSHNQLQSLPLLGQTLPALTVLDVSFNRLTSLPLGALRGLGELQELYLKGNELKTLPPGLLTPTPKLEKLSLANNNLTELPAGLLNGLENLDTLLLQENSLYTIPKGFFGSHLLPFAFLHGNPWLCNCEILYFRRWLQDNAENVYVWKQVVDVKAVTSNVASVQCDNSDKFPVYKYPGKGCPTLGDEGDTDLYDYYPEEDTEGDKVR

SEQ ID NO: 43 - protein, 8 aa, Synthetic
HHHHHHHH

SEQ ID NO: 44 - protein, 9 aa, Synthetic
GHHHHHHHH

SEQ ID NO: 45 - protein, 27 aa, Synthetic
EEDTEDYKDHDGDYKDHDIDYKDDDDK

SEQ ID NO: 46 - protein, 236 aa, Synthetic
VPRDCGCKPCICTVPEVSSVFIFPPKPKDVLTITLTPKVTCVVVDISKDDPEVQFSWFVDDVEVHTAQTQPREEQFNSTFRSVSELPIMHQDWLNGKEFKCRVNSAAFPAPIEKTISKTKGRPKAPQVYTIPPPKEQMAKDKVSLTCMITDFFPEDITVEWQWNGQPAENYKNTQPIMDTDGSYFVYSKLNVQKSNWEAGNTFTCSVLHEGLHNHHTEKSLSHSPGIGHHHHHHHH